European Patent Specification EP 3 969 605 B1, published November 20, 2024. Title: Methods. Applicant: Phoremost Limited. The sequence listing filed with the application follows.

SEQUENCE LISTING (10 sequences)

SEQ ID NO: 1 - protein, 16 aa, Artificial Sequence
  Target protein binding moiety peptide
LPHLQRSPPDGQSFRS

SEQ ID NO: 2 - protein, 7 aa, Artificial Sequence
  E3 ligase binding moeity peptide
ALAPYIP

SEQ ID NO: 3 - protein, 6 aa, Artificial Sequence
  GGGGSS Linker
GGGGSS

SEQ ID NO: 4 - protein, 34 aa, Artificial Sequence
  3BP2(410-425)- ALAPYIP peptide
MGLPHLQRSPPDGQSFRSLEGGGGSSAALAPYIP

SEQ ID NO: 5 - protein, 26 aa, Artificial Sequence
  3BP2(410-425) linker peptide
MGLPHLQRSPPDGQSFRSLEGGGGSS

SEQ ID NO: 6 - protein, 34 aa, Artificial Sequence
  3BP2(410-425)- ALAAAIP peptide
MGLPHLQRSPPDGQSFRSLEGGGGSSAALAAAIP

SEQ ID NO: 7 - protein, 35 aa, Artificial Sequence
  3BP2(410-425) - LDPETGEYL peptide
MGLPHLQRSPPDGQSFRSLEGGGGSSLDPETGEYL

SEQ ID NO: 8 - protein, 317 aa, Artificial Sequence
  E3 reporter peptide
MATKDQLFPLAKEFIDQYYSSIKKFGSKAHMERLEEVNKEIDTTSGGGSRVSKGEELFTGVVPILVELDGDVNGHKFSVSGEGEGDATYGKLTLKFICTTGKLPVPWPTLVTTFTYGVQCFARYPDHMKQHDFFKSAMPEGYVQERTIFFKDDGNYKTRAEVKFEGDTLVNRIELKGIDFKEDGNILGHKLEYNYNSHKVYITADKQKNGIKVNFKTRHNIEDGSVQLADHYQQNTPIGDGPVLLPDNHYLSTQSALSKDPNEKRDHMVLLEFVTAAGITLGMDELYKEFGGGSAIHAVLTSINQSSIALAGSSAAT

SEQ ID NO: 9 - protein, 11 aa, Artificial Sequence
  HIF1 alpha VHL binding sequence
LDLEMLAPYIP

SEQ ID NO: 10 - protein, 46 aa, Artificial Sequence
  Candidate peptide
MQNNPLTSGLEPSPPQCDYIRPSLTGKFAGNPWYYGKVTRHQAEMA